European Patent Application EP 4 768 584 A1, published July 1, 2026. Title: 用于抑制二酰甘油-O-酰基转移酶2表达的RNAi剂及其应用. Applicant: 云合智药（苏州）生物科技有限公司. The sequence listing filed with the application follows.

SEQUENCE LISTING (64 sequences)

SEQ ID NO: 1 - RNA, 19 nt, synthetic construct
  source 1..19: mol_type = other RNA
agaagaagttccagaaata

SEQ ID NO: 2 - RNA, 19 nt, synthetic construct
  source 1..19: mol_type = other RNA
ggctcatcgctgtgctcta

SEQ ID NO: 3 - RNA, 19 nt, synthetic construct
  source 1..19: mol_type = other RNA
agcaagacatcgacctgta

SEQ ID NO: 4 - RNA, 19 nt, synthetic construct
  source 1..19: mol_type = other RNA
gagagaatgaagtgtacaa

SEQ ID NO: 5 - RNA, 19 nt, synthetic construct
  source 1..19: mol_type = other RNA
tggtgaagctcttcgacaa

SEQ ID NO: 6 - RNA, 19 nt, synthetic construct
  source 1..19: mol_type = other RNA
ggaggtatctgccctgtca

SEQ ID NO: 7 - RNA, 19 nt, synthetic construct
  source 1..19: mol_type = other RNA
ctactttcgagactacttt

SEQ ID NO: 8 - RNA, 19 nt, synthetic construct
  source 1..19: mol_type = other RNA
ggaactatatctttggata

SEQ ID NO: 9 - RNA, 19 nt, synthetic construct
  source 1..19: mol_type = other RNA
ggcgctactttcgagacta

SEQ ID NO: 10 - RNA, 19 nt, synthetic construct
  source 1..19: mol_type = other RNA
gctccatgcctggcaagaa

SEQ ID NO: 11 - RNA, 19 nt, synthetic construct
  source 1..19: mol_type = other RNA
tctgtcacctggctcaata

SEQ ID NO: 12 - RNA, 19 nt, synthetic construct
  source 1..19: mol_type = other RNA
ggttatttaaaagaaatta

SEQ ID NO: 13 - RNA, 19 nt, synthetic construct
  source 1..19: mol_type = other RNA
gtctgtgggttatttaaaa

SEQ ID NO: 14 - RNA, 19 nt, synthetic construct
  source 1..19: mol_type = other RNA
gtaaatttggaagtgtcat

SEQ ID NO: 15 - RNA, 19 nt, synthetic construct
  source 1..19: mol_type = other RNA
ctactttcgagactacttt

SEQ ID NO: 16 - RNA, 19 nt, synthetic construct
  source 1..19: mol_type = other RNA
atagactatttgctttcaa

SEQ ID NO: 17 - RNA, 21 nt, synthetic construct
  source 1..21: mol_type = other RNA
tatttctggaacttcttctgg

SEQ ID NO: 18 - RNA, 21 nt, synthetic construct
  source 1..21: mol_type = other RNA
tagagcacagcgatgagccag

SEQ ID NO: 19 - RNA, 21 nt, synthetic construct
  source 1..21: mol_type = other RNA
tacaggtcgatgtcttgctgg

SEQ ID NO: 20 - RNA, 21 nt, synthetic construct
  source 1..21: mol_type = other RNA
ttgtacacttcattctctcca

SEQ ID NO: 21 - RNA, 21 nt, synthetic construct
  source 1..21: mol_type = other RNA
ttgtcgaagagcttcaccagg

SEQ ID NO: 22 - RNA, 21 nt, synthetic construct
  source 1..21: mol_type = other RNA
tgacagggcagatacctccag

SEQ ID NO: 23 - RNA, 21 nt, synthetic construct
  source 1..21: mol_type = other RNA
aaagtagtctcgaaagtagcg

SEQ ID NO: 24 - RNA, 21 nt, synthetic construct
  source 1..21: mol_type = other RNA
tatccaaagatatagttcctg

SEQ ID NO: 25 - RNA, 21 nt, synthetic construct
  source 1..21: mol_type = other RNA
tagtctcgaaagtagcgccac

SEQ ID NO: 26 - RNA, 21 nt, synthetic construct
  source 1..21: mol_type = other RNA
ttcttgccaggcatggagctc

SEQ ID NO: 27 - RNA, 21 nt, synthetic construct
  source 1..21: mol_type = other RNA
tattgagccaggtgacagaga

SEQ ID NO: 28 - RNA, 21 nt, synthetic construct
  source 1..21: mol_type = other RNA
taatttcttttaaataaccca

SEQ ID NO: 29 - RNA, 21 nt, synthetic construct
  source 1..21: mol_type = other RNA
ttttaaataacccacagacac

SEQ ID NO: 30 - RNA, 21 nt, synthetic construct
  source 1..21: mol_type = other RNA
atgacacttccaaatttacag

SEQ ID NO: 31 - RNA, 19 nt, synthetic construct
  source 1..19: mol_type = other RNA
ctactttcgagactacttt

SEQ ID NO: 32 - RNA, 21 nt, synthetic construct
  source 1..21: mol_type = other RNA
ttgaaagcaaatagtctatgg

SEQ ID NO: 33 - RNA, 19 nt, synthetic construct
  source 1..19: mol_type = other RNA
agaagaagttccagaaata

SEQ ID NO: 34 - RNA, 21 nt, synthetic construct
  source 1..21: mol_type = other RNA
tatttctggaacttcttctgg

SEQ ID NO: 35 - RNA, 21 nt, synthetic construct
  source 1..21: mol_type = other RNA
tatttctggaacttcttctgg

SEQ ID NO: 36 - RNA, 21 nt, synthetic construct
  source 1..21: mol_type = other RNA
tatttctggaacttcttctgg

SEQ ID NO: 37 - RNA, 19 nt, synthetic construct
  source 1..19: mol_type = other RNA
agaagaagttccagaaata

SEQ ID NO: 38 - RNA, 19 nt, synthetic construct
  source 1..19: mol_type = other RNA
ggctcatcgctgtgctcta

SEQ ID NO: 39 - RNA, 21 nt, synthetic construct
  source 1..21: mol_type = other RNA
tagagcacagcgatgagccag

SEQ ID NO: 40 - RNA, 21 nt, synthetic construct
  source 1..21: mol_type = other RNA
tagagcacagcgatgagccag

SEQ ID NO: 41 - RNA, 21 nt, synthetic construct
  source 1..21: mol_type = other RNA
tagagcacagcgatgagccag

SEQ ID NO: 42 - RNA, 19 nt, synthetic construct
  source 1..19: mol_type = other RNA
ggctcatcgctgtgctcta

SEQ ID NO: 43 - RNA, 19 nt, synthetic construct
  source 1..19: mol_type = other RNA
ggcgctactttcgagacta

SEQ ID NO: 44 - RNA, 21 nt, synthetic construct
  source 1..21: mol_type = other RNA
tagtctcgaaagtagcgccac

SEQ ID NO: 45 - RNA, 21 nt, synthetic construct
  source 1..21: mol_type = other RNA
tagtctcgaaagtagcgccac

SEQ ID NO: 46 - RNA, 21 nt, synthetic construct
  source 1..21: mol_type = other RNA
tagtctcgaaagtagcgccac

SEQ ID NO: 47 - RNA, 19 nt, synthetic construct
  source 1..19: mol_type = other RNA
ggcgctactttcgagacta

SEQ ID NO: 48 - RNA, 19 nt, synthetic construct
  source 1..19: mol_type = other RNA
atagactatttgctttcaa

SEQ ID NO: 49 - RNA, 21 nt, synthetic construct
  source 1..21: mol_type = other RNA
ttgaaagcaaatagtctatgg

SEQ ID NO: 50 - RNA, 19 nt, synthetic construct
  source 1..19: mol_type = other RNA
agaagaagttccagaaata

SEQ ID NO: 51 - RNA, 19 nt, synthetic construct
  source 1..19: mol_type = other RNA
agaagaagttccagaaata

SEQ ID NO: 52 - RNA, 19 nt, synthetic construct
  source 1..19: mol_type = other RNA
ggctcatcgctgtgctcta

SEQ ID NO: 53 - RNA, 19 nt, synthetic construct
  source 1..19: mol_type = other RNA
ggctcatcgctgtgctcta

SEQ ID NO: 54 - RNA, 19 nt, synthetic construct
  source 1..19: mol_type = other RNA
ggcgctactttcgagacta

SEQ ID NO: 55 - RNA, 19 nt, synthetic construct
  source 1..19: mol_type = other RNA
tggtgaagctcttcgacaa

SEQ ID NO: 56 - RNA, 21 nt, synthetic construct
  source 1..21: mol_type = other RNA
ttgtcgaagagcttcaccagg

SEQ ID NO: 57 - RNA, 21 nt, synthetic construct
  source 1..21: mol_type = other RNA
ttgtcgaagagcttcaccagg

SEQ ID NO: 58 - RNA, 21 nt, synthetic construct
  source 1..21: mol_type = other RNA
ttgtcgaagagcttcaccagg

SEQ ID NO: 59 - RNA, 19 nt, synthetic construct
  source 1..19: mol_type = other RNA
ctactttcgagactacttt

SEQ ID NO: 60 - RNA, 21 nt, synthetic construct
  source 1..21: mol_type = other RNA
aaagtagtctcgaaagtagcg

SEQ ID NO: 61 - RNA, 21 nt, synthetic construct
  source 1..21: mol_type = other RNA
aaagtagtctcgaaagtagcg

SEQ ID NO: 62 - RNA, 21 nt, synthetic construct
  source 1..21: mol_type = other RNA
aaagtagtctcgaaagtagcg

SEQ ID NO: 63 - RNA, 19 nt, synthetic construct
  source 1..19: mol_type = other RNA
atagactatttgctttcaa

SEQ ID NO: 64 - RNA, 19 nt, synthetic construct
  source 1..19: mol_type = other RNA
tggtgaagctcttcgacaa